European Patent Application EP 4 170 034 A1, published April 26, 2023. Title: NOVEL TRANSGLUTAMINASE. Applicant: AMANO ENZYME INC. THE UNIVERSITY OF TOKYO. The sequence listing filed with the application follows.

SEQUENCE LISTING (6 sequences)

SEQ ID NO: 1 - protein, 697 aa, Aspergillus oryzae
MAEETQVLSIQQRIAALNQAQVGQSPQAAASPLLGAQPTPFASRPAPSRQQTINNPPVNSHDSLGDRNEPTGAQPKPVPRPPPIPVQKPRAPPPLPARKASTESAPALPPRRPSGFSRKESRESLGSDVSHSTSTSAGRATIASTTSNNSDTIRSVRAPAWGAKLPPLPPKRQDTKTVQPPPRPRPSPANSSRSLSQGRPSLPPRRESTNSTSTNGNRSTSRPPPPLPSRINSDKSPGPSADTNGKQSTRKLPPPPPSSAALEKIQSSGLAGINRNTENSGKGTNGSVQEPQPNGVPPPVPRATRPDVDLAKLQATKPRLCKTTHSATAPSTMCLKCRDFSAPDAHAAQYPRESLPSYDLAWLARELTAPFPSPTDKARALFTWFHHNIEYDVHSFFNKCVKPSTPAGTLASGLAVCEGYASLFATLATHAGLEAVVVAGHGKGYGYDAPAPGSPIPPVSATGHAWSAVRIDNGQWKLLDACWGAGVVQGPGLPYKKQFNPAMFTDSNDEFGLRHFPSNRSHFFRDDGRPEITWEEYILGNPNSPLSAEQPTIFGDAQNHSIGERSFRPAAKQISIHDPSPLRFQFNLICEHWTLEHHTRAKPGLFLLMVHGLDGRQDDRLPFTHVRGSGPGGGGDFWYVDVPNAKILGAPGQKLAIAVLTSFGDRKDARGVTAEEYRQQVGRVGMAWAYIAEWQLV

SEQ ID NO: 2 - protein, 339 aa, Aspergillus oryzae
DLAWLARELTAPFPSPTDKARALFTWFHHNIEYDVHSFFNKCVKPSTPAGTLASGLAVCEGYASLFATLATHAGLEAVVVAGHGKGYGYDAPAPGSPIPPVSATGHAWSAVRIDNGQWKLLDACWGAGVVQGPGLPYKKQFNPAMFTDSNDEFGLRHFPSNRSHFFRDDGRPEITWEEYILGNPNSPLSAEQPTIFGDAQNHSIGERSFRPAAKQISIHDPSPLRFQFNLICEHWTLEHHTRAKPGLFLLMVHGLDGRQDDRLPFTHVRGSGPGGGGDFWYVDVPNAKILGAPGQKLAIAVLTSFGDRKDARGVTAEEYRQQVGRVGMAWAYIAEWQLV

SEQ ID NO: 3 - protein, 123 aa, Aspergillus oryzae
DLAWLARELTAPFPSPTDKARALFTWFHHNIEYDVHSFFNKCVKPSTPAGTLASGLAVCEGYASLFATLATHAGLEAVVVAGHGKGYGYDAPAPGSPIPPVSATGHAWSAVRIDNGQWKLLDA

SEQ ID NO: 4 - DNA, 2094 bp, Aspergillus oryzae
atggcagaagagacacaggtcctttccatccagcaacggatcgccgccctgaaccaggcgcaggtcggacaaagccctcaggctgccgcatccccgttactcggggcgcaaccaacccctttcgcatcgcgtccagccccttcgcgacagcaaacgatcaataatcctccagtcaattcccatgactctcttggtgatagaaacgagccaaccggggcgcaaccaaaacctgtgcccaggccaccaccaatacctgttcagaaaccaagggcccctccaccgttgccggctcgaaaggcgtcaactgaatcagcaccagcgctaccaccacgaagaccgtcagggttctctcgaaaggaatctagggagtccctaggctcggatgtgtcccattcaacgtctacaagtgcggggagggctacaatagcatcgaccacgtctaataactcggataccatccgcagtgtacgtgcgcctgcatggggtgcaaaattgcctcctttgccaccgaaaagacaagatacgaaaaccgttcaaccgcccccacgaccgagaccatcacctgcaaatagcagcagaagcctctcgcagggtcgcccctcactaccccctcggcgagagtcgaccaacagcacgtcaactaatggaaaccgctctacctctcggcctcctccgccattaccttctagaataaatagcgacaagtcacctggaccaagtgcagacacaaatggcaagcaatcaacgagaaaattgccaccgccgcccccctcgagtgctgctctggagaagattcaaagttcagggcttgcagggataaaccggaacaccgagaactctgggaaagggacgaatggtagtgtacaagagccgcagccgaacggggtgccacccccagttcccagagcgacacgtccagatgtcgacctcgccaaacttcaggcgactaaacctcgcctttgtaaaaccacgcattcagctacggcaccgagcacaatgtgcttgaagtgccgcgatttctcggcgcctgatgctcatgcagcgcaatatcctcgcgagtcactgccgtcttacgacttggcatggctggcgagggaactgacagcgccgtttccttcccccactgataaagcgagggccttgttcacttggttccaccataatatagaatacgatgtgcattccttcttcaacaaatgtgtaaaaccttccacgccagcgggaactctagcgtcaggactggcggtgtgtgaaggatacgccagtctatttgcaactctcgcaacccacgctgggctcgaggcggtagtagtcgctggtcacggcaagggctatggctatgacgctccagctccaggctcccccataccaccggtttcggcaaccggacatgcctggagtgcagtgaggattgataatggacagtggaagctgttggacgcctgttggggtgcaggtgtagttcagggtccaggcctcccttacaagaagcaatttaacccggccatgttcaccgactcgaatgacgagttcgggctccgacatttcccttccaaccgatctcacttcttccgggatgatggccggcccgagatcacttgggaggagtacatcctgggcaacccgaactcaccattgagtgctgagcagccgacaatctttggcgacgcacaaaaccacagcataggcgaacggtcattccgtccggcggccaagcaaatctccatccacgaccccagcccgctccggttccagttcaatctcatctgcgaacactggaccctggagcatcacacccgagctaagcctgggcttttcttgctgatggttcacggcctcgacggtcggcaagacgaccgtctccccttcacccatgtccggggctccggaccggggggaggcggggacttctggtatgtcgatgtaccgaatgccaagatactgggtgcacccggtcagaagctagccatcgccgtacttaccagcttcggggatcgaaaggacgcacggggcgtgaccgcggaagaatatcggcagcaagtcggtcgggtaggaatggcgtgggcgtacattgcggagtggcagctggtgtga

SEQ ID NO: 5 - DNA, 1020 bp, Aspergillus oryzae
gacttggcatggctggcgagggaactgacagcgccgtttccttcccccactgataaagcgagggccttgttcacttggttccaccataatatagaatacgatgtgcattccttcttcaacaaatgtgtaaaaccttccacgccagcgggaactctagcgtcaggactggcggtgtgtgaaggatacgccagtctatttgcaactctcgcaacccacgctgggctcgaggcggtagtagtcgctggtcacggcaagggctatggctatgacgctccagctccaggctcccccataccaccggtttcggcaaccggacatgcctggagtgcagtgaggattgataatggacagtggaagctgttggacgcctgttggggtgcaggtgtagttcagggtccaggcctcccttacaagaagcaatttaacccggccatgttcaccgactcgaatgacgagttcgggctccgacatttcccttccaaccgatctcacttcttccgggatgatggccggcccgagatcacttgggaggagtacatcctgggcaacccgaactcaccattgagtgctgagcagccgacaatctttggcgacgcacaaaaccacagcataggcgaacggtcattccgtccggcggccaagcaaatctccatccacgaccccagcccgctccggttccagttcaatctcatctgcgaacactggaccctggagcatcacacccgagctaagcctgggcttttcttgctgatggttcacggcctcgacggtcggcaagacgaccgtctccccttcacccatgtccggggctccggaccggggggaggcggggacttctggtatgtcgatgtaccgaatgccaagatactgggtgcacccggtcagaagctagccatcgccgtacttaccagcttcggggatcgaaaggacgcacggggcgtgaccgcggaagaatatcggcagcaagtcggtcgggtaggaatggcgtgggcgtacattgcggagtggcagctggtgtga

SEQ ID NO: 6 - DNA, 369 bp, Aspergillus oryzae
gacttggcatggctggcgagggaactgacagcgccgtttccttcccccactgataaagcgagggccttgttcacttggttccaccataatatagaatacgatgtgcattccttcttcaacaaatgtgtaaaaccttccacgccagcgggaactctagcgtcaggactggcggtgtgtgaaggatacgccagtctatttgcaactctcgcaacccacgctgggctcgaggcggtagtagtcgctggtcacggcaagggctatggctatgacgctccagctccaggctcccccataccaccggtttcggcaaccggacatgcctggagtgcagtgaggattgataatggacagtggaagctgttggacgcc